European Patent Application EP 4 763 867 A1, published June 24, 2026. Title: PHARMACEUTICAL COMPOSITION CONTAINING IMMUNOCONJUGATE AND USE THEREOF. Applicant: Shanghai MabGen Biotech Ltd. Application WO PCT/CN2024/112330, filed August 15, 2024. The sequence listing filed with the application follows.

SEQUENCE LISTING (50 sequences)

SEQ ID NO: 1 - protein, 288 aa, Synthetic Construct
MQIPQAPWPVVWAVLQLGWRPGWFLDSPDRPWNPPTFSPALLVVTEGDNATFTCSFSNTSESFVLNWYRMSPSNQTDKLAAFPEDRSQPGQDCRFRVTQLPNGRDFHMSVVRARRNDSGTYLCGAISLAPKAQIKESLRAELRVTERRAEVPTAHPSPSPRPAGQFQTLVVGVVGGLLGSLVLLVWVLAVICSRAARGTIGARRTGQPLKEDPSAVPVFSVDYGELDFQWREKTPEPPVPCVPEQTEYATIVFPSGMGTSSPARRGSADGPRSAQPLRPEDGHCSWPL

SEQ ID NO: 2 - protein, 116 aa, Synthetic Construct
EVQVVESGGGLVQPGGSLRLSCVASGLTFSDYSMSWYRQAPGKERELVAIISGSGVIAHYVDSVKGRFTISRDNAKSTVYLQMVSLKPEDRGVYYCRAVSDWDDYWGQGTQVTVSS

SEQ ID NO: 3 - protein, 5 aa, Synthetic Construct
DYSMS

SEQ ID NO: 4 - protein, 17 aa, Synthetic Construct
IISGSGVIAHYVDSVKG

SEQ ID NO: 5 - protein, 7 aa, Synthetic Construct
VSDWDDY

SEQ ID NO: 6 - protein, 229 aa, Synthetic Construct
ESKYGPPCPPCPAPEFLGGPSVFLFPPKPKDTLMISRTPEVTCVVVDVSQEDPEVQFNWYVDGVEVHNAKTKPREEQFNSTYRVVSVLTVLHQDWLNGKEYKCKVSNKGLPSSIEKTISKAKGQPREPQVYTLPPSQEEMTKNQVSLTCLVKGFYPSDIAVEWESNGQPENNYKTTPPVLDSDGSFFLYSRLTVDKSRWQEGNVFSCSVMHEALHNHYTQKSLSLSLGK

SEQ ID NO: 7 - protein, 345 aa, Synthetic Construct
EVQVVESGGGLVQPGGSLRLSCVASGLTFSDYSMSWYRQAPGKERELVAIISGSGVIAHYVDSVKGRFTISRDNAKSTVYLQMVSLKPEDRGVYYCRAVSDWDDYWGQGTQVTVSSESKYGPPCPPCPAPEFLGGPSVFLFPPKPKDTLMISRTPEVTCVVVDVSQEDPEVQFNWYVDGVEVHNAKTKPREEQFNSTYRVVSVLTVLHQDWLNGKEYKCKVSNKGLPSSIEKTISKAKGQPREPQVYTLPPSQEEMTKNQVSLTCLVKGFYPSDIAVEWESNGQPENNYKTTPPVLDSDGSFFLYSRLTVDKSRWQEGNVFSCSVMHEALHNHYTQKSLSLSLGK

SEQ ID NO: 8 - protein, 116 aa, Synthetic Construct
EVQLQESGGGLVQPGGSLRLSCTASGLTFSDYSMSWYRQAPGKGRELVAIISGSGVIAHYVDSVKGRFTISRDNSKNTVYLQMRSLTPEDRAVYYCRAVSDWDDYWGQGTQVTVSS

SEQ ID NO: 9 - protein, 116 aa, Synthetic Construct
EVQLVESGGGLVQPGGSLRLSCAASGLTFSDYSMSWVRQAPGKGLEWVAIISGSGVIAHYVDSVKGRFTISRDNSKNTVYLQMNSLRAEDTAVYYCRAVSDWDDYWGQGTQVTVSS

SEQ ID NO: 10 - protein, 116 aa, Synthetic Construct
EVQLVESGGGLVQPGGSLRLSCAASGLTFSDYSMSWVRQAPGKGLEWVAIISGSGVIAHYVDSVKGRFTISRDNSKNTVYLQMNSLRAEDTAVYYCRAVSDWDEYWGQGTQVTVSS

SEQ ID NO: 11 - protein, 115 aa, Synthetic Construct
EVQLQESGGGLVQPGGSLRLSCTASGLTFSDYSMSWYRQAPGKGRELVAIISGSGVITHYVDSVKGRTISRDNAKNTVYLQMRSLTPEDRAVYYCRAVSDWEDYWGQGTQVTVSS

SEQ ID NO: 12 - protein, 116 aa, Synthetic Construct
EVQLVESGGGLVQPGGSLRLSCAASGFTFSDYSMSWYRQAPGKGRELVAIISGSGVITHYVDSVKGRFTISRDNAKNTLYLQMRSLRAEDTAVYYCRAVSDWEDYWGQGTQVTVSS

SEQ ID NO: 13 - protein, 116 aa, Synthetic Construct
EVQLVESGGGLVQPGGSLRLSCAASGLTFSDYSMSWYRQAPGKGRELVAIISGSGVITHYVDSVKGRFTISRDNAKNTLYLQMRSLRAEDTAVYYCRAVSDWEDYWGQGTQVTVSS

SEQ ID NO: 14 - protein, 116 aa, Synthetic Construct
EVQLVESGGGLVQPGGSLRLSCAASGLTFSDYSMSWYRQAPGKGRELVAIISGSGVITHYVDSVKGRFTISRDNAKNTVYLQMRSLRAEDTAVYYCRAVSDWEDYWGQGTQVTVSS

SEQ ID NO: 15 - protein, 116 aa, Synthetic Construct
EVQLVESGGGLVQPGGSLRLSCAASGLTFSDYSMSWYRQAPGKGRELVAIISGSGVITHYVDSVKGRFTISRDNAKNTVYLQMRSLRAEDRAVYYCRAVSDWEDYWGQGTQVTVSS

SEQ ID NO: 16 - protein, 17 aa, Synthetic Construct
  VARIANT 9: note; note (original language) = X is selected from the group consisting of T and A
IISGSGVIXHYVDSVKG

SEQ ID NO: 17 - protein, 7 aa, Synthetic Construct
  VARIANT 5: note; note (original language) = X is selected from the group consisting of D and E
  VARIANT 6: note; note (original language) = X is selected from the group consisting of D and E
VSDWXXY

SEQ ID NO: 18 - protein, 17 aa, Synthetic Construct
IISGSGVITHYVDSVKG

SEQ ID NO: 19 - protein, 7 aa, Synthetic Construct
VSDWEDY

SEQ ID NO: 20 - protein, 7 aa, Synthetic Construct
VSDWDEY

SEQ ID NO: 21 - protein, 495 aa, Synthetic Construct
EVQLQESGGGLVQPGGSLRLSCTASGLTFSDYSMSWYRQAPGKGRELVAIISGSGVIAHYVDSVKGRFTISRDNSKNTVYLQMRSLTPEDRAVYYCRAVSDWDDYWGQGTQVTVSSEPKSSDKTHTCPPCPAPEAAGGPSVFLFPPKPKDTLMISRTPEVTCVVVDVSHEDPEVKFNWYVDGVEVHNAKTKPREEQYNSTYRVVSVLTVLHQDWLNGKEYKCKVSNKALGAPIEKTISKAKGQPREPQVYTLPPCRDELTKNQVSLWCLVKGFYPSDIAVEWESNGQPENNYKTTPPVLDSDGSFFLYSKLTVDKSRWQQGNVFSCSVMHEALHNHYTQKSLSLSPGGGGGSGGGGSGGGGSAPASSSTKKTQLQLEHLLLDLQMILNGINNYKNPKLTEMLTAKFYMPKKATELKHLQCLEEELKPLEEVLNLAQSKNFHLRPRDLISNINTIVLELKGSETTFMCEYADETATIVEFLNRWITFAQSIISTLT

SEQ ID NO: 22 - protein, 346 aa, Synthetic Construct
EVQLQESGGGLVQPGGSLRLSCTASGLTFSDYSMSWYRQAPGKGRELVAIISGSGVIAHYVDSVKGRFTISRDNSKNTVYLQMRSLTPEDRAVYYCRAVSDWDDYWGQGTQVTVSSEPKSSDKTHTCPPCPAPEAAGGPSVFLFPPKPKDTLMISRTPEVTCVVVDVSHEDPEVKFNWYVDGVEVHNAKTKPREEQYNSTYRVVSVLTVLHQDWLNGKEYKCKVSNKALGAPIEKTISKAKGQPREPQVCTLPPSRDELTKNQVSLSCAVKGFYPSDIAVEWESNGQPENNYKTTPPVLDSDGSFFLVSKLTVDKSRWQQGNVFSCSVMHEALHNRFTQKSLSLSP

SEQ ID NO: 23 - protein, 133 aa, Synthetic Construct
APASSSTKKTQLQLEHLLLDLQMILNGINNYKNPKLTEMLTAKFYMPKKATELKHLQCLEEELKPLEEVLNLAQSKNFHLRPRDLISNINTIVLELKGSETTFMCEYADETATIVEFLNRWITFAQSIISTLT

SEQ ID NO: 24 - protein, 133 aa, Synthetic Construct
APASSSTKKTQLQLEHLLLDLQMILQGISNYKNPKLTRMLTAKFYMPKKATELKHLQCLEEELKPLEEVLQGAQSKNFHLRPRDLISNINVIVLELKGSETTFMCEYADETATIVEFLNRWITFAQSIISTLT

SEQ ID NO: 25 - protein, 133 aa, Synthetic Construct
APASSSTKKTQLQLEHLLLDLQMILQGISNYKNPKLTRMLTAKFYMPKKATELKHLQCLEEELKPLEEVLQGAQSKNFHLRPRDLISNINTIVLELKGSETTFMCEYADETATIVEFLNRWITFAQSIISTLT

SEQ ID NO: 26 - protein, 133 aa, Synthetic Construct
APASSSTKKTQLQLEHLLLALQMILQGISNYKNPKLTRMLTAKFYMPKKATELKHLQCLEEELKPLEEVLQGAQSKNFHLRPRDLISNINVIVLELKGSETTFMCEYADETATIVEFLNRWITFAQSIISTLT

SEQ ID NO: 27 - protein, 133 aa, Synthetic Construct
APASSSTKKTQLQLEHLLLNLQMILQGISNYKNPKLTRMLTAKFYMPKKATELKHLQCLEEELKPLEEVLQGAQSKNFHLRPRDLISNINVIVLELKGSETTFMCEYADETATIVEFLNRWITFAQSIISTLT

SEQ ID NO: 28 - protein, 133 aa, Synthetic Construct
APASSSTKKTQLQLEHLLLDLQMILQGISNYKNPKLTRMLTAKFYMPKKATELKHLQCLEEELKPLEEVLQGAQSKNFHLRPRDLISDINVIVLELKGSETTFMCEYADETATIVEFLNRWITFAQSIISTLT

SEQ ID NO: 29 - protein, 133 aa, Synthetic Construct
APASSSTKKTQLQLEHLLLDLQMILQGISNYKNPKLTRMLTAKFYMPKKATELKHLQCLEEELKPLEEVLQGAQSKNFHLRPRDLISRINVIVLELKGSETTFMCEYADETATIVEFLNRWITFAQSIISTLT

SEQ ID NO: 30 - protein, 133 aa, Synthetic Construct
APASSSTKKTQLQLEHLLLDLQMILQGISNYKNPKLTRMLTAKFYMPKKATELKHLQCLEEELKPLEEVLQGAQSKNFHLRPRDLISNINVIVLELKGSETTFMCEYADETATIVEFLNRWITFADSIISTLT

SEQ ID NO: 31 - protein, 133 aa, Synthetic Construct
APASSSTKKTQLQLEALLLDLQMILQGISNYKNPKLTRMLTAKFYMPKKATELKHLQCLEEELKPLEEVLQGAQSKNFHLRPRSLISNINVIVLELKGSETTFMCEYADETATIVEFLNRWITFAQSIISTLT

SEQ ID NO: 32 - protein, 231 aa, Synthetic Construct
EPKSSDKTHTCPPCPAPEAAGGPSVFLFPPKPKDTLMISRTPEVTCVVVDVSHEDPEVKFNWYVDGVEVHNAKTKPREEQYNSTYRVVSVLTVLHQDWLNGKEYKCKVSNKALPAPIEKTISKAKGQPREPQVYTLPPCRDELTKNQVSLWCLVKGFYPSDIAVEWESNGQPENNYKTTPPVLDSDGSFFLYSKLTVDKSRWQQGNVFSCSVMHEALHNHYTQKSLSLSPG

SEQ ID NO: 33 - protein, 230 aa, Synthetic Construct
EPKSSDKTHTCPPCPAPEAAGGPSVFLFPPKPKDTLMISRTPEVTCVVVDVSHEDPEVKFNWYVDGVEVHNAKTKPREEQYNSTYRVVSVLTVLHQDWLNGKEYKCKVSNKALPAPIEKTISKAKGQPREPQVCTLPPSRDELTKNQVSLSCAVKGFYPSDIAVEWESNGQPENNYKTTPPVLDSDGSFFLVSKLTVDKSRWQQGNVFSCSVMHEALHNHYTQKSLSLSP

SEQ ID NO: 34 - protein, 231 aa, Synthetic Construct
EPKSSDKTHTCPPCPAPEAAGGPSVFLFPPKPKDTLMISRTPEVTCVVVDVSHEDPEVKFNWYVDGVEVHNAKTKPREEQYNSTYRVVSVLTVLHQDWLNGKEYKCKVSNKALPAPIEKTISKAKGQPREPQVYTLPPCREEMTKNQVSLWCLVKGFYPSDIAVEWESNGQPENNYKTTPPVLDSDGSFFLYSKLTVDKSRWQQGNVFSCSVMHEALHNHYTQKSLSLSPG

SEQ ID NO: 35 - protein, 231 aa, Synthetic Construct
EPKSSDKTHTCPPCPAPEAAGGPSVFLFPPKPKDTLMISRTPEVTCVVVDVSHEDPEVKFNWYVDGVEVHNAKTKPREEQYNSTYRVVSVLTVLHQDWLNGKEYKCKVSNKALPAPIEKTISKAKGQPREPQVCTLPPSREEMTKNQVSLSCAVKGFYPSDIAVEWESNGQPENNYKTTPPVLDSDGSFFLVSKLTVDKSRWQQGNVFSCSVMHEALHNHYTQKSLSLSPG

SEQ ID NO: 36 - protein, 495 aa, Synthetic Construct
EVQLVESGGGLVQPGGSLRLSCAASGLTFSDYSMSWYRQAPGKGRELVAIISGSGVITHYVDSVKGRFTISRDNAKNTLYLQMRSLRAEDTAVYYCRAVSDWEDYWGQGTQVTVSSEPKSSDKTHTCPPCPAPEAAGGPSVFLFPPKPKDTLMISRTPEVTCVVVDVSHEDPEVKFNWYVDGVEVHNAKTKPREEQYNSTYRVVSVLTVLHQDWLNGKEYKCKVSNKALPAPIEKTISKAKGQPREPQVYTLPPCRDELTKNQVSLWCLVKGFYPSDIAVEWESNGQPENNYKTTPPVLDSDGSFFLYSKLTVDKSRWQQGNVFSCSVMHEALHNHYTQKSLSLSPGGGGGSGGGGSGGGGSAPASSSTKKTQLQLEHLLLALQMILQGISNYKNPKLTRMLTAKFYMPKKATELKHLQCLEEELKPLEEVLQGAQSKNFHLRPRDLISNINVIVLELKGSETTFMCEYADETATIVEFLNRWITFAQSIISTLT

SEQ ID NO: 37 - protein, 346 aa, Synthetic Construct
EVQLVESGGGLVQPGGSLRLSCAASGLTFSDYSMSWYRQAPGKGRELVAIISGSGVITHYVDSVKGRFTISRDNAKNTLYLQMRSLRAEDTAVYYCRAVSDWEDYWGQGTQVTVSSEPKSSDKTHTCPPCPAPEAAGGPSVFLFPPKPKDTLMISRTPEVTCVVVDVSHEDPEVKFNWYVDGVEVHNAKTKPREEQYNSTYRVVSVLTVLHQDWLNGKEYKCKVSNKALPAPIEKTISKAKGQPREPQVCTLPPSRDELTKNQVSLSCAVKGFYPSDIAVEWESNGQPENNYKTTPPVLDSDGSFFLVSKLTVDKSRWQQGNVFSCSVMHEALHNRFTQKSLSLSP

SEQ ID NO: 38 - protein, 495 aa, Synthetic Construct
EVQLVESGGGLVQPGGSLRLSCAASGLTFSDYSMSWYRQAPGKGRELVAIISGSGVITHYVDSVKGRFTISRDNAKNTLYLQMRSLRAEDTAVYYCRAVSDWEDYWGQGTQVTVSSEPKSSDKTHTCPPCPAPEAAGGPSVFLFPPKPKDTLMISRTPEVTCVVVDVSHEDPEVKFNWYVDGVEVHNAKTKPREEQYNSTYRVVSVLTVLHQDWLNGKEYKCKVSNKALPAPIEKTISKAKGQPREPQVYTLPPCREEMTKNQVSLWCLVKGFYPSDIAVEWESNGQPENNYKTTPPVLDSDGSFFLYSKLTVDKSRWQQGNVFSCSVMHEALHNHYTQKSLSLSPGGGGGSGGGGSGGGGSAPASSSTKKTQLQLEHLLLALQMILQGISNYKNPKLTRMLTAKFYMPKKATELKHLQCLEEELKPLEEVLQGAQSKNFHLRPRDLISNINVIVLELKGSETTFMCEYADETATIVEFLNRWITFAQSIISTLT

SEQ ID NO: 39 - protein, 347 aa, Synthetic Construct
EVQLVESGGGLVQPGGSLRLSCAASGLTFSDYSMSWYRQAPGKGRELVAIISGSGVITHYVDSVKGRFTISRDNAKNTLYLQMRSLRAEDTAVYYCRAVSDWEDYWGQGTQVTVSSEPKSSDKTHTCPPCPAPEAAGGPSVFLFPPKPKDTLMISRTPEVTCVVVDVSHEDPEVKFNWYVDGVEVHNAKTKPREEQYNSTYRVVSVLTVLHQDWLNGKEYKCKVSNKALPAPIEKTISKAKGQPREPQVCTLPPSREEMTKNQVSLSCAVKGFYPSDIAVEWESNGQPENNYKTTPPVLDSDGSFFLVSKLTVDKSRWQQGNVFSCSVMHEALHNHYTQKSLSLSPG

SEQ ID NO: 40 - protein, 495 aa, Synthetic Construct
EVQLVESGGGLVQPGGSLRLSCAASGLTFSDYSMSWYRQAPGKGRELVAIISGSGVITHYVDSVKGRFTISRDNAKNTLYLQMRSLRAEDTAVYYCRAVSDWEDYWGQGTQVTVSSEPKSSDKTHTCPPCPAPEAAGGPSVFLFPPKPKDTLMISRTPEVTCVVVDVSHEDPEVKFNWYVDGVEVHNAKTKPREEQYNSTYRVVSVLTVLHQDWLNGKEYKCKVSNKALPAPIEKTISKAKGQPREPQVYTLPPCRDELTKNQVSLWCLVKGFYPSDIAVEWESNGQPENNYKTTPPVLDSDGSFFLYSKLTVDKSRWQQGNVFSCSVMHEALHNHYTQKSLSLSPGGGGGSGGGGSGGGGSAPASSSTKKTQLQLEHLLLDLQMILQGISNYKNPKLTRMLTAKFYMPKKATELKHLQCLEEELKPLEEVLQGAQSKNFHLRPRDLISDINVIVLELKGSETTFMCEYADETATIVEFLNRWITFAQSIISTLT

SEQ ID NO: 41 - protein, 346 aa, Synthetic Construct
EVQLVESGGGLVQPGGSLRLSCAASGLTFSDYSMSWYRQAPGKGRELVAIISGSGVITHYVDSVKGRFTISRDNAKNTLYLQMRSLRAEDTAVYYCRAVSDWEDYWGQGTQVTVSSEPKSSDKTHTCPPCPAPEAAGGPSVFLFPPKPKDTLMISRTPEVTCVVVDVSHEDPEVKFNWYVDGVEVHNAKTKPREEQYNSTYRVVSVLTVLHQDWLNGKEYKCKVSNKALPAPIEKTISKAKGQPREPQVCTLPPSRDELTKNQVSLSCAVKGFYPSDIAVEWESNGQPENNYKTTPPVLDSDGSFFLVSKLTVDKSRWQQGNVFSCSVMHEALHNHYTQKSLSLSP

SEQ ID NO: 42 - protein, 495 aa, Synthetic Construct
EVQLVESGGGLVQPGGSLRLSCAASGLTFSDYSMSWYRQAPGKGRELVAIISGSGVITHYVDSVKGRFTISRDNAKNTLYLQMRSLRAEDTAVYYCRAVSDWEDYWGQGTQVTVSSEPKSSDKTHTCPPCPAPEAAGGPSVFLFPPKPKDTLMISRTPEVTCVVVDVSHEDPEVKFNWYVDGVEVHNAKTKPREEQYNSTYRVVSVLTVLHQDWLNGKEYKCKVSNKALPAPIEKTISKAKGQPREPQVYTLPPCREEMTKNQVSLWCLVKGFYPSDIAVEWESNGQPENNYKTTPPVLDSDGSFFLYSKLTVDKSRWQQGNVFSCSVMHEALHNHYTQKSLSLSPGGGGGSGGGGSGGGGSAPASSSTKKTQLQLEHLLLDLQMILQGISNYKNPKLTRMLTAKFYMPKKATELKHLQCLEEELKPLEEVLQGAQSKNFHLRPRDLISDINVIVLELKGSETTFMCEYADETATIVEFLNRWITFAQSIISTLT

SEQ ID NO: 43 - protein, 347 aa, Synthetic Construct; identical to SEQ ID NO: 39

SEQ ID NO: 44 - protein, 595 aa, Synthetic Construct
QVQLVQSGAEVKKPGASVKVSCKASGYTFTNSWIGWFRQAPGQGLEWIGDIYPGGGYTNYNEIFKGKATMTADTSTNTAYMELSSLRSEDTAVYYCSRGIPGYAMDYWGQGTLVTVSSASTKGPSVFPLAPSSKSTSGGTAALGCLVKDYFPEPVTVSWNSGALTSGVHTFPAVLQSSGLYSLSSVVTVPSSSLGTQTYICNVNHKPSNTKVDKKVEPKSCDKTHTCPPCPAPEAAGGPSVFLFPPKPKDTLMISRTPEVTCVVVDVSHEDPEVKFNWYVDGVEVHNAKTKPREEQYNSTYRVVSVLTVLHQDWLNGKEYKCKVSNKALGAPIEKTISKAKGQPREPQVYTLPPCRDELTKNQVSLWCLVKGFYPSDIAVEWESNGQPENNYKTTPPVLDSDGSFFLYSKLTVDKSRWQQGNVFSCSVMHEALHNHYTQKSLSLSPGGGGGSGGGGSGGGGSAPASSSTKKTQLQLEHLLLDLQMILQGISNYKNPKLTRMLTAKFYMPKKATELKHLQCLEEELKPLEEVLQGAQSKNFHLRPRDLISNINVIVLELKGSETTFMCEYADETATIVEFLNRWITFAQSIISTLT

SEQ ID NO: 45 - protein, 595 aa, Synthetic Construct
QVQLVQSGAEVKKPGASVKVSCKASGYTFTNSWIGWFRQAPGQGLEWIGDIYPGGGYTNYNEIFKGKATMTADTSTNTAYMELSSLRSEDTAVYYCSRGIPGYAMDYWGQGTLVTVSSASTKGPSVFPLAPSSKSTSGGTAALGCLVKDYFPEPVTVSWNSGALTSGVHTFPAVLQSSGLYSLSSVVTVPSSSLGTQTYICNVNHKPSNTKVDKKVEPKSCDKTHTCPPCPAPEAAGGPSVFLFPPKPKDTLMISRTPEVTCVVVDVSHEDPEVKFNWYVDGVEVHNAKTKPREEQYNSTYRVVSVLTVLHQDWLNGKEYKCKVSNKALGAPIEKTISKAKGQPREPQVYTLPPCRDELTKNQVSLWCLVKGFYPSDIAVEWESNGQPENNYKTTPPVLDSDGSFFLYSKLTVDKSRWQQGNVFSCSVMHEALHNHYTQKSLSLSPGGGGGSGGGGSGGGGSAPASSSTKKTQLQLEHLLLDLQMILNGINNYKNPKLTEMLTAKFYMPKKATELKHLQCLEEELKPLEEVLNLAQSKNFHLRPRDLISNINTIVLELKGSETTFMCEYADETATIVEFLNRWITFAQSIISTLT

SEQ ID NO: 46 - protein, 595 aa, Synthetic Construct
QVQLVQSGAEVKKPGASVKVSCKASGYTFTNSWIGWFRQAPGQGLEWIGDIYPGGGYTNYNEIFKGKATMTADTSTNTAYMELSSLRSEDTAVYYCSRGIPGYAMDYWGQGTLVTVSSASTKGPSVFPLAPSSKSTSGGTAALGCLVKDYFPEPVTVSWNSGALTSGVHTFPAVLQSSGLYSLSSVVTVPSSSLGTQTYICNVNHKPSNTKVDKKVEPKSCDKTHTCPPCPAPEAAGGPSVFLFPPKPKDTLMISRTPEVTCVVVDVSHEDPEVKFNWYVDGVEVHNAKTKPREEQYNSTYRVVSVLTVLHQDWLNGKEYKCKVSNKALGAPIEKTISKAKGQPREPQVYTLPPCRDELTKNQVSLWCLVKGFYPSDIAVEWESNGQPENNYKTTPPVLDSDGSFFLYSKLTVDKSRWQQGNVFSCSVMHEALHNHYTQKSLSLSPGGGGGSGGGGSGGGGSAPASSSTKKTQLQLEHLLLDLQMILQGISNYKNPKLTRMLTAKFYMPKKATELKHLQCLEEELKPLEEVLQGAQSKNFHLRPRDLISDINVIVLELKGSETTFMCEYADETATIVEFLNRWITFAQSIISTLT

SEQ ID NO: 47 - protein, 595 aa, Synthetic Construct
QVQLVQSGAEVKKPGASVKVSCKASGYTFTNSWIGWFRQAPGQGLEWIGDIYPGGGYTNYNEIFKGKATMTADTSTNTAYMELSSLRSEDTAVYYCSRGIPGYAMDYWGQGTLVTVSSASTKGPSVFPLAPSSKSTSGGTAALGCLVKDYFPEPVTVSWNSGALTSGVHTFPAVLQSSGLYSLSSVVTVPSSSLGTQTYICNVNHKPSNTKVDKKVEPKSCDKTHTCPPCPAPEAAGGPSVFLFPPKPKDTLMISRTPEVTCVVVDVSHEDPEVKFNWYVDGVEVHNAKTKPREEQYNSTYRVVSVLTVLHQDWLNGKEYKCKVSNKALGAPIEKTISKAKGQPREPQVYTLPPCRDELTKNQVSLWCLVKGFYPSDIAVEWESNGQPENNYKTTPPVLDSDGSFFLYSKLTVDKSRWQQGNVFSCSVMHEALHNHYTQKSLSLSPGGGGGSGGGGSGGGGSAPASSSTKKTQLQLEHLLLALQMILQGISNYKNPKLTRMLTAKFYMPKKATELKHLQCLEEELKPLEEVLQGAQSKNFHLRPRDLISNINVIVLELKGSETTFMCEYADETATIVEFLNRWITFAQSIISTLT

SEQ ID NO: 48 - protein, 446 aa, Synthetic Construct
QVQLVQSGAEVKKPGASVKVSCKASGYTFTNSWIGWFRQAPGQGLEWIGDIYPGGGYTNYNEIFKGKATMTADTSTNTAYMELSSLRSEDTAVYYCSRGIPGYAMDYWGQGTLVTVSSASTKGPSVFPLAPSSKSTSGGTAALGCLVKDYFPEPVTVSWNSGALTSGVHTFPAVLQSSGLYSLSSVVTVPSSSLGTQTYICNVNHKPSNTKVDKKVEPKSCDKTHTCPPCPAPEAAGGPSVFLFPPKPKDTLMISRTPEVTCVVVDVSHEDPEVKFNWYVDGVEVHNAKTKPREEQYNSTYRVVSVLTVLHQDWLNGKEYKCKVSNKALGAPIEKTISKAKGQPREPQVCTLPPSRDELTKNQVSLSCAVKGFYPSDIAVEWESNGQPENNYKTTPPVLDSDGSFFLVSKLTVDKSRWQQGNVFSCSVMHEALHNRFTQKSLSLSP

SEQ ID NO: 49 - protein, 220 aa, Synthetic Construct
DIQMTQSPSSLSASVGDRVTMSCKSSQSLLNSGDQKNYLTWYQQKPGKAPKLLIYWASTGESGVPSRFSGSGSGTDFTFTISSLQPEDIATYYCQNDYSYPWTFGQGTKVEIKRTVAAPSVFIFPPSDEQLKSGTASVVCLLNNFYPREAKVQWKVDNALQSGNSQESVTEQDSKDSTYSLSSTLTLSKADYEKHKVYACEVTHQGLSSPVTKSFNRGEC

SEQ ID NO: 50 - protein, 133 aa, Synthetic Construct [sequence omitted]